European Patent Specification EP 3 743 091 B1, published November 6, 2024. Title: METHODS AND COMPOSITIONS FOR TREATMENT OF ANGIOGENIC DISORDERS USING ANTI-VEGF AGENTS. Applicant: THE REGENTS OF THE UNIVERSITY OF CALIFORNIA. The sequence listing filed with the application follows.

SEQUENCE LISTING (14 sequences)

SEQ ID NO: 1 - protein, 558 aa, Artificial Sequence
  Description of Artificial Sequence: Synthetic polypeptide
MVSYWDTGVLLCALLSCLLLTGSSSGSKLKDPELSLKGTQHIMQAGQTLHLQCRGEAAHKWSLPEMVSKESERLSITKSACGRNGKQFCSTLTLNTAQANHTGFYSCKYLAVPTSKKKETESAIYIFISDTGRPFVEMYSEIPEIIHMTEGRELVIPCRVTSPNITVTLKKFPLDTLIPDGKRIIWDSRKGFIISNATYKEIGLLTCEATVNGHLYKTNYLTHRQTNTIIDVQISTPRPVKLLRGHTLVLNCTATTPLNTRVQMTWSYPDEKNKRASVRRRIDQSNSHANIFYSVLTIDKMQNKDKGLYTCRVRSGPSFKSVNTSVHIYDKDKTHTCPPCPAPELLGGPSVFLFPPKPKDTLMISRTPEVTCVVVDVSHEDPEVKFNWYVDGVEVHNAKTKPREEQYNSTYRVVSVLTVLHQDWLNGKEYKCKVSNKALPAPIEKTISKAKGQPREPQVYTLPPSREEMTKNQVSLTCLVKGFYPSDIAVEWESNGQPENNYKTTPPVLDSDGSFFLYSKLTVDKSRWQQGNVFSCSVMHEALHNHYTQKSLSLSPGK

SEQ ID NO: 2 - DNA, 1674 bp, Artificial Sequence
  Description of Artificial Sequence: Synthetic polynucleotide
atggtcagctactgggacaccggggtcctgctgtgcgcgctgctcagctgtctgcttctcacaggatctagttcaggttcaaaattaaaagatcctgaactgagtttaaaaggcacccagcacatcatgcaagcaggccagacactgcatctccaatgcaggggggaagcagcccataaatggtctttgcctgaaatggtgagtaaggaaagcgaaaggctgagcataactaaatctgcctgtggaagaaatggcaaacaattctgcagtactttaaccttgaacacagctcaagcaaaccacactggcttctacagctgcaaatatctagctgtacctacttcaaagaagaaggaaacagaatctgcaatctatatatttattagtgatacaggtagacctttcgtagagatgtacagtgaaatccccgaaattatacacatgactgaaggaagggagctcgtcattccctgccgggttacgtcacctaacatcactgttactttaaaaaagtttccacttgacactttgatccctgatggaaaacgcataatctgggacagtagaaagggcttcatcatatcaaatgcaacgtacaaagaaatagggcttctgacctgtgaagcaacagtcaatgggcatttgtataagacaaactatctcacacatcgacaaaccaatacaatcatagatgtccaaataagcacaccacgcccagtcaaattacttagaggccatactcttgtcctcaattgtactgctaccactcccttgaacacgagagttcaaatgacctggagttaccctgatgaaaaaaataagagagcttccgtaaggcgacgaattgaccaaagcaattcccatgccaacatattctacagtgttcttactattgacaaaatgcagaacaaagacaaaggactttatacttgtcgtgtaaggagtggaccatcattcaaatctgttaacacctcagtgcatatatatgataaagacaaaactcacacatgcccaccgtgcccagcacctgaactcctggggggaccgtcagtcttcctcttccccccaaaacccaaggacaccctcatgatctcccggacccctgaggtcacatgcgtggtggtggacgtgagccacgaagaccctgaggtcaagttcaactggtacgtggacggcgtggaggtgcataatgccaagacaaagccgcgggaggagcagtacaacagcacgtaccgtgtggtcagcgtcctcaccgtcctgcaccaggactggctgaatggcaaggagtacaagtgcaaggtctccaacaaagccctcccagcccccatcgagaaaaccatctccaaagccaaagggcagccccgagaaccacaggtgtacaccctgcccccatcccgggaggagatgaccaagaaccaggtcagcctgacctgcctggtcaaaggcttctatcccagcgacatcgccgtggagtgggagagcaatgggcagccggagaacaactacaagaccacgcctcccgtgctggactccgacggctccttcttcctctacagcaagctcaccgtggacaagagcaggtggcagcaggggaacgtcttctcatgctccgtgatgcacgaggctctgcacaaccactacacgcagaagagcctctccctgtctccgggtaaa

SEQ ID NO: 3 - protein, 459 aa, Artificial Sequence
  Description of Artificial Sequence: Synthetic polypeptide
MVSYWDTGVLLCALLSCLLLTGSSSGIFISDTGRPFVEMYSEIPEIIHMTEGRELVIPCRVTSPNITVTLKKFPLDTLIPDGKRIIWDSRKGFIISNATYKEIGLLTCEATVNGHLYKTNYLTHRQTNTIIDVQISTPRPVKLLRGHTLVLNCTATTPLNTRVQMTWSYPDEKNKRASVRRRIDQSNSHANIFYSVLTIDKMQNKDKGLYTCRVRSGPSFKSVNTSVHIYDKDKTHTCPPCPAPELLGGPSVFLFPPKPKDTLMISRTPEVTCVVVDVSHEDPEVKFNWYVDGVEVHNAKTKPREEQYNSTYRVVSVLTVLHQDWLNGKEYKCKVSNKALPAPIEKTISKAKGQPREPQVYTLPPSREEMTKNQVSLTCLVKGFYPSDIAVEWESNGQPENNYKTTPPVLDSDGSFFLYSKLTVDKSRWQQGNVFSCSVMHEALHNHYTQKSLSLSPGK

SEQ ID NO: 4 - DNA, 1377 bp, Artificial Sequence
  Description of Artificial Sequence: Synthetic polynucleotide
atggtcagctactgggacaccggggtcctgctgtgcgcgctgctcagctgtctgcttctcacaggatctagttcaggtatatttattagtgatacaggtagacctttcgtagagatgtacagtgaaatccccgaaattatacacatgactgaaggaagggagctcgtcattccctgccgggttacgtcacctaacatcactgttactttaaaaaagtttccacttgacactttgatccctgatggaaaacgcataatctgggacagtagaaagggcttcatcatatcaaatgcaacgtacaaagaaatagggcttctgacctgtgaagcaacagtcaatgggcatttgtataagacaaactatctcacacatcgacaaaccaatacaatcatagatgtccaaataagcacaccacgcccagtcaaattacttagaggccatactcttgtcctcaattgtactgctaccactcccttgaacacgagagttcaaatgacctggagttaccctgatgaaaaaaataagagagcttccgtaaggcgacgaattgaccaaagcaattcccatgccaacatattctacagtgttcttactattgacaaaatgcagaacaaagacaaaggactttatacttgtcgtgtaaggagtggaccatcattcaaatctgttaacacctcagtgcatatatatgataaagacaaaactcacacatgcccaccgtgcccagcacctgaactcctggggggaccgtcagtcttcctcttccccccaaaacccaaggacaccctcatgatctcccggacccctgaggtcacatgcgtggtggtggacgtgagccacgaagaccctgaggtcaagttcaactggtacgtggacggcgtggaggtgcataatgccaagacaaagccgcgggaggagcagtacaacagcacgtaccgtgtggtcagcgtcctcaccgtcctgcaccaggactggctgaatggcaaggagtacaagtgcaaggtctccaacaaagccctcccagcccccatcgagaaaaccatctccaaagccaaagggcagccccgagaaccacaggtgtacaccctgcccccatcccgggaggagatgaccaagaaccaggtcagcctgacctgcctggtcaaaggcttctatcccagcgacatcgccgtggagtgggagagcaatgggcagccggagaacaactacaagaccacgcctcccgtgctggactccgacggctccttcttcctctacagcaagctcaccgtggacaagagcaggtggcagcaggggaacgtcttctcatgctccgtgatgcacgaggctctgcacaaccactacacgcagaagagcctctccctgtctccgggtaaa

SEQ ID NO: 5 - protein, 659 aa, Artificial Sequence
  Description of Artificial Sequence: Synthetic polypeptide
MVSYWDTGVLLCALLSCLLLTGSSSGSKLKDPELSLKGTQHIMQAGQTLHLQCRGEAAHKWSLPEMVSKESERLSITKSACGRNGKQFCSTLTLNTAQANHTGFYSCKYLAVPTSKKKETESAIYIFISDTGRPFVEMYSEIPEIIHMTEGRELVIPCRVTSPNITVTLKKFPLDTLIPDGKRIIWDSRKGFIISNATYKEIGLLTCEATVNGHLYKTNYLTHRQTNTIIDVQISTPRPVKLLRGHTLVLNCTATTPLNTRVQMTWSYPDEKNKRASVRRRIDQSNSHANIFYSVLTIDKMQNKDKGLYTCRVRSGPSFKSVNTSVHIYDKAVQISTPRPVKLLRGHTLVLNCTATTPLNTRVQMTWSYPDEKNKRASVRRRIDQSNSHANIFYSVLTIDKMQNKDKGLYTCRVRSGPSFKSVNTSVHIYDKDKTHTCPPCPAPELLGGPSVFLFPPKPKDTLMISRTPEVTCVVVDVSHEDPEVKFNWYVDGVEVHNAKTKPREEQYNSTYRVVSVLTVLHQDWLNGKEYKCKVSNKALPAPIEKTISKAKGQPREPQVYTLPPSREEMTKNQVSLTCLVKGFYPSDIAVEWESNGQPENNYKTTPPVLDSDGSFFLYSKLTVDKSRWQQGNVFSCSVMHEALHNHYTQKSLSLSPGK

SEQ ID NO: 6 - DNA, 1977 bp, Artificial Sequence
  Description of Artificial Sequence: Synthetic polynucleotide
atggtcagctactgggacaccggggtcctgctgtgcgcgctgctcagctgtctgcttctcacaggatctagttcaggttcaaaattaaaagatcctgaactgagtttaaaaggcacccagcacatcatgcaagcaggccagacactgcatctccaatgcaggggggaagcagcccataaatggtctttgcctgaaatggtgagtaaggaaagcgaaaggctgagcataactaaatctgcctgtggaagaaatggcaaacaattctgcagtactttaaccttgaacacagctcaagcaaaccacactggcttctacagctgcaaatatctagctgtacctacttcaaagaagaaggaaacagaatctgcaatctatatatttattagtgatacaggtagacctttcgtagagatgtacagtgaaatccccgaaattatacacatgactgaaggaagggagctcgtcattccctgccgggttacgtcacctaacatcactgttactttaaaaaagtttccacttgacactttgatccctgatggaaaacgcataatctgggacagtagaaagggcttcatcatatcaaatgcaacgtacaaagaaatagggcttctgacctgtgaagcaacagtcaatgggcatttgtataagacaaactatctcacacatcgacaaaccaatacaatcatagatgtccaaataagcacaccacgcccagtcaaattacttagaggccatactcttgtcctcaattgtactgctaccactcccttgaacacgagagttcaaatgacctggagttaccctgatgaaaaaaataagagagcttccgtaaggcgacgaattgaccaaagcaattcccatgccaacatattctacagtgttcttactattgacaaaatgcagaacaaagacaaaggactttatacttgtcgtgtaaggagtggaccatcattcaaatctgttaacacctcagtgcatatatatgataaagcagtccaaataagcacaccacgcccagtcaaattacttagaggccatactcttgtcctcaattgtactgctaccactcccttgaacacgagagttcaaatgacctggagttaccctgatgaaaaaaataagagagcttccgtaaggcgacgaattgaccaaagcaattcccatgccaacatattctacagtgttcttactattgacaaaatgcagaacaaagacaaaggactttatacttgtcgtgtaaggagtggaccatcattcaaatctgttaacacctcagtgcatatatatgataaagacaaaactcacacatgcccaccgtgcccagcacctgaactcctggggggaccgtcagtcttcctcttccccccaaaacccaaggacaccctcatgatctcccggacccctgaggtcacatgcgtggtggtggacgtgagccacgaagaccctgaggtcaagttcaactggtacgtggacggcgtggaggtgcataatgccaagacaaagccgcgggaggagcagtacaacagcacgtaccgtgtggtcagcgtcctcaccgtcctgcaccaggactggctgaatggcaaggagtacaagtgcaaggtctccaacaaagccctcccagcccccatcgagaaaaccatctccaaagccaaagggcagccccgagaaccacaggtgtacaccctgcccccatcccgggaggagatgaccaagaaccaggtcagcctgacctgcctggtcaaaggcttctatcccagcgacatcgccgtggagtgggagagcaatgggcagccggagaacaactacaagaccacgcctcccgtgctggactccgacggctccttcttcctctacagcaagctcaccgtggacaagagcaggtggcagcaggggaacgtcttctcatgctccgtgatgcacgaggctctgcacaaccactacacgcagaagagcctctccctgtctccgggtaaa

SEQ ID NO: 7 - protein, 560 aa, Artificial Sequence
  Description of Artificial Sequence: Synthetic polypeptide
MVSYWDTGVLLCALLSCLLLTGSSSGIFISDTGRPFVEMYSEIPEIIHMTEGRELVIPCRVTSPNITVTLKKFPLDTLIPDGKRIIWDSRKGFIISNATYKEIGLLTCEATVNGHLYKTNYLTHRQTNTIIDVQISTPRPVKLLRGHTLVLNCTATTPLNTRVQMTWSYPDEKNKRASVRRRIDQSNSHANIFYSVLTIDKMQNKDKGLYTCRVRSGPSFKSVNTSVHIYDKAVQISTPRPVKLLRGHTLVLNCTATTPLNTRVQMTWSYPDEKNKRASVRRRIDQSNSHANIFYSVLTIDKMQNKDKGLYTCRVRSGPSFKSVNTSVHIYDKDKTHTCPPCPAPELLGGPSVFLFPPKPKDTLMISRTPEVTCVVVDVSHEDPEVKFNWYVDGVEVHNAKTKPREEQYNSTYRVVSVLTVLHQDWLNGKEYKCKVSNKALPAPIEKTISKAKGQPREPQVYTLPPSREEMTKNQVSLTCLVKGFYPSDIAVEWESNGQPENNYKTTPPVLDSDGSFFLYSKLTVDKSRWQQGNVFSCSVMHEALHNHYTQKSLSLSPGK

SEQ ID NO: 8 - DNA, 1680 bp, Artificial Sequence
  Description of Artificial Sequence: Synthetic polynucleotide
atggtcagctactgggacaccggggtcctgctgtgcgcgctgctcagctgtctgcttctcacaggatctagttcaggtatatttattagtgatacaggtagacctttcgtagagatgtacagtgaaatccccgaaattatacacatgactgaaggaagggagctcgtcattccctgccgggttacgtcacctaacatcactgttactttaaaaaagtttccacttgacactttgatccctgatggaaaacgcataatctgggacagtagaaagggcttcatcatatcaaatgcaacgtacaaagaaatagggcttctgacctgtgaagcaacagtcaatgggcatttgtataagacaaactatctcacacatcgacaaaccaatacaatcatagatgtccaaataagcacaccacgcccagtcaaattacttagaggccatactcttgtcctcaattgtactgctaccactcccttgaacacgagagttcaaatgacctggagttaccctgatgaaaaaaataagagagcttccgtaaggcgacgaattgaccaaagcaattcccatgccaacatattctacagtgttcttactattgacaaaatgcagaacaaagacaaaggactttatacttgtcgtgtaaggagtggaccatcattcaaatctgttaacacctcagtgcatatatatgataaagcagtccaaataagcacaccacgcccagtcaaattacttagaggccatactcttgtcctcaattgtactgctaccactcccttgaacacgagagttcaaatgacctggagttaccctgatgaaaaaaataagagagcttccgtaaggcgacgaattgaccaaagcaattcccatgccaacatattctacagtgttcttactattgacaaaatgcagaacaaagacaaaggactttatacttgtcgtgtaaggagtggaccatcattcaaatctgttaacacctcagtgcatatatatgataaagacaaaactcacacatgcccaccgtgcccagcacctgaactcctggggggaccgtcagtcttcctcttccccccaaaacccaaggacaccctcatgatctcccggacccctgaggtcacatgcgtggtggtggacgtgagccacgaagaccctgaggtcaagttcaactggtacgtggacggcgtggaggtgcataatgccaagacaaagccgcgggaggagcagtacaacagcacgtaccgtgtggtcagcgtcctcaccgtcctgcaccaggactggctgaatggcaaggagtacaagtgcaaggtctccaacaaagccctcccagcccccatcgagaaaaccatctccaaagccaaagggcagccccgagaaccacaggtgtacaccctgcccccatcccgggaggagatgaccaagaaccaggtcagcctgacctgcctggtcaaaggcttctatcccagcgacatcgccgtggagtgggagagcaatgggcagccggagaacaactacaagaccacgcctcccgtgctggactccgacggctccttcttcctctacagcaagctcaccgtggacaagagcaggtggcagcaggggaacgtcttctcatgctccgtgatgcacgaggctctgcacaaccactacacgcagaagagcctctccctgtctccgggtaaa

SEQ ID NO: 9 - protein, 655 aa, Artificial Sequence
  Description of Artificial Sequence: Synthetic polypeptide
MVSYWDTGVLLCALLSCLLLTGSSSGSKLKDPELSLKGTQHIMQAGQTLHLQCRGEAAHKWSLPEMVSKESERLSITKSACGRNGKQFCSTLTLNTAQANHTGFYSCKYLAVPTSKKKETESAIYIFISDTGRPFVEMYSEIPEIIHMTEGRELVIPCRVTSPNITVTLKKFPLDTLIPDGKRIIWDSRKGFIISNATYKEIGLLTCEATVNGHLYKTNYLTHRQTNTIIDVQISTPRPVKLLRGHTLVLNCTATTPLNTRVQMTWSYPDEKNKRASVRRRIDQSNSHANIFYSVLTIDKMQNKDKGLYTCRVRSGPSFKSVNTSVHIYDKAFITVKHRKQQVLETVAGKRSYRLSMKVKAFPSPEVVWLKDGLPATEKSARYLTRGYSLIIKDVTEEDAGNYTILLSIKQSNVFKNLTATLIVNVKPDKTHTCPPCPAPELLGGPSVFLFPPKPKDTLMISRTPEVTCVVVDVSHEDPEVKFNWYVDGVEVHNAKTKPREEQYNSTYRVVSVLTVLHQDWLNGKEYKCKVSNKALPAPIEKTISKAKGQPREPQVYTLPPSREEMTKNQVSLTCLVKGFYPSDIAVEWESNGQPENNYKTTPPVLDSDGSFFLYSKLTVDKSRWQQGNVFSCSVMHEALHNHYTQKSLSLSPGK

SEQ ID NO: 10 - DNA, 1965 bp, Artificial Sequence
  Description of Artificial Sequence: Synthetic polynucleotide
atggtcagctactgggacaccggggtcctgctgtgcgcgctgctcagctgtctgcttctcacaggatctagttcaggttcaaaattaaaagatcctgaactgagtttaaaaggcacccagcacatcatgcaagcaggccagacactgcatctccaatgcaggggggaagcagcccataaatggtctttgcctgaaatggtgagtaaggaaagcgaaaggctgagcataactaaatctgcctgtggaagaaatggcaaacaattctgcagtactttaaccttgaacacagctcaagcaaaccacactggcttctacagctgcaaatatctagctgtacctacttcaaagaagaaggaaacagaatctgcaatctatatatttattagtgatacaggtagacctttcgtagagatgtacagtgaaatccccgaaattatacacatgactgaaggaagggagctcgtcattccctgccgggttacgtcacctaacatcactgttactttaaaaaagtttccacttgacactttgatccctgatggaaaacgcataatctgggacagtagaaagggcttcatcatatcaaatgcaacgtacaaagaaatagggcttctgacctgtgaagcaacagtcaatgggcatttgtataagacaaactatctcacacatcgacaaaccaatacaatcatagatgtccaaataagcacaccacgcccagtcaaattacttagaggccatactcttgtcctcaattgtactgctaccactcccttgaacacgagagttcaaatgacctggagttaccctgatgaaaaaaataagagagcttccgtaaggcgacgaattgaccaaagcaattcccatgccaacatattctacagtgttcttactattgacaaaatgcagaacaaagacaaaggactttatacttgtcgtgtaaggagtggaccatcattcaaatctgttaacacctcagtgcatatatatgataaagcattcatcactgtgaaacatcgaaaacagcaggtgcttgaaaccgtagctggcaagcggtcttaccggctctctatgaaagtgaaggcatttccctcgccggaagttgtatggttaaaagatgggttacctgcgactgagaaatctgctcgctatttgactcgtggctactcgttaattatcaaggacgtaactgaagaggatgcagggaattatacaatcttgctgagcataaaacagtcaaatgtgtttaaaaacctcactgccactctaattgtcaatgtgaaacccgacaaaactcacacatgcccaccgtgcccagcacctgaactcctggggggaccgtcagtcttcctcttccccccaaaacccaaggacaccctcatgatctcccggacccctgaggtcacatgcgtggtggtggacgtgagccacgaagaccctgaggtcaagttcaactggtacgtggacggcgtggaggtgcataatgccaagacaaagccgcgggaggagcagtacaacagcacgtaccgtgtggtcagcgtcctcaccgtcctgcaccaggactggctgaatggcaaggagtacaagtgcaaggtctccaacaaagccctcccagcccccatcgagaaaaccatctccaaagccaaagggcagccccgagaaccacaggtgtacaccctgcccccatcccgggaggagatgaccaagaaccaggtcagcctgacctgcctggtcaaaggcttctatcccagcgacatcgccgtggagtgggagagcaatgggcagccggagaacaactacaagaccacgcctcccgtgctggactccgacggctccttcttcctctacagcaagctcaccgtggacaagagcaggtggcagcaggggaacgtcttctcatgctccgtgatgcacgaggctctgcacaaccactacacgcagaagagcctctccctgtctccgggtaaa

SEQ ID NO: 11 - protein, 556 aa, Artificial Sequence
  Description of Artificial Sequence: Synthetic polypeptide
MVSYWDTGVLLCALLSCLLLTGSSSGIFISDTGRPFVEMYSEIPEIIHMTEGRELVIPCRVTSPNITVTLKKFPLDTLIPDGKRIIWDSRKGFIISNATYKEIGLLTCEATVNGHLYKTNYLTHRQTNTIIDVQISTPRPVKLLRGHTLVLNCTATTPLNTRVQMTWSYPDEKNKRASVRRRIDQSNSHANIFYSVLTIDKMQNKDKGLYTCRVRSGPSFKSVNTSVHIYDKAFITVKHRKQQVLETVAGKRSYRLSMKVKAFPSPEVVWLKDGLPATEKSARYLTRGYSLIIKDVTEEDAGNYTILLSIKQSNVFKNLTATLIVNVKPDKTHTCPPCPAPELLGGPSVFLFPPKPKDTLMISRTPEVTCVVVDVSHEDPEVKFNWYVDGVEVHNAKTKPREEQYNSTYRVVSVLTVLHQDWLNGKEYKCKVSNKALPAPIEKTISKAKGQPREPQVYTLPPSREEMTKNQVSLTCLVKGFYPSDIAVEWESNGQPENNYKTTPPVLDSDGSFFLYSKLTVDKSRWQQGNVFSCSVMHEALHNHYTQKSLSLSPGK

SEQ ID NO: 12 - DNA, 1668 bp, Artificial Sequence
  Description of Artificial Sequence: Synthetic polynucleotide
atggtcagctactgggacaccggggtcctgctgtgcgcgctgctcagctgtctgcttctcacaggatctagttcaggtatatttattagtgatacaggtagacctttcgtagagatgtacagtgaaatccccgaaattatacacatgactgaaggaagggagctcgtcattccctgccgggttacgtcacctaacatcactgttactttaaaaaagtttccacttgacactttgatccctgatggaaaacgcataatctgggacagtagaaagggcttcatcatatcaaatgcaacgtacaaagaaatagggcttctgacctgtgaagcaacagtcaatgggcatttgtataagacaaactatctcacacatcgacaaaccaatacaatcatagatgtccaaataagcacaccacgcccagtcaaattacttagaggccatactcttgtcctcaattgtactgctaccactcccttgaacacgagagttcaaatgacctggagttaccctgatgaaaaaaataagagagcttccgtaaggcgacgaattgaccaaagcaattcccatgccaacatattctacagtgttcttactattgacaaaatgcagaacaaagacaaaggactttatacttgtcgtgtaaggagtggaccatcattcaaatctgttaacacctcagtgcatatatatgataaagcattcatcactgtgaaacatcgaaaacagcaggtgcttgaaaccgtagctggcaagcggtcttaccggctctctatgaaagtgaaggcatttccctcgccggaagttgtatggttaaaagatgggttacctgcgactgagaaatctgctcgctatttgactcgtggctactcgttaattatcaaggacgtaactgaagaggatgcagggaattatacaatcttgctgagcataaaacagtcaaatgtgtttaaaaacctcactgccactctaattgtcaatgtgaaacccgacaaaactcacacatgcccaccgtgcccagcacctgaactcctggggggaccgtcagtcttcctcttccccccaaaacccaaggacaccctcatgatctcccggacccctgaggtcacatgcgtggtggtggacgtgagccacgaagaccctgaggtcaagttcaactggtacgtggacggcgtggaggtgcataatgccaagacaaagccgcgggaggagcagtacaacagcacgtaccgtgtggtcagcgtcctcaccgtcctgcaccaggactggctgaatggcaaggagtacaagtgcaaggtctccaacaaagccctcccagcccccatcgagaaaaccatctccaaagccaaagggcagccccgagaaccacaggtgtacaccctgcccccatcccgggaggagatgaccaagaaccaggtcagcctgacctgcctggtcaaaggcttctatcccagcgacatcgccgtggagtgggagagcaatgggcagccggagaacaactacaagaccacgcctcccgtgctggactccgacggctccttcttcctctacagcaagctcaccgtggacaagagcaggtggcagcaggggaacgtcttctcatgctccgtgatgcacgaggctctgcacaaccactacacgcagaagagcctctccctgtctccgggtaaa

SEQ ID NO: 13 - protein, 456 aa, Artificial Sequence
  Description of Artificial Sequence: Synthetic polypeptide
MVSYWDTGVLLCALLSCLLLTGSSSGIFISDTGRPFVEMYSEIPEIIHMTEGRELVIPCRVTSPNITVTLKKFPLDTLIPDGKRIIWDSRKGFIISNATYKEIGLLTCEATVNGHLYKTNYLTHRQTNTIIDVFITVKHRKQQVLETVAGKRSYRLSMKVKAFPSPEVVWLKDGLPATEKSARYLTRGYSLIIKDVTEEDAGNYTILLSIKQSNVFKNLTATLIVNVKPDKTHTCPPCPAPELLGGPSVFLFPPKPKDTLMISRTPEVTCVVVDVSHEDPEVKFNWYVDGVEVHNAKTKPREEQYNSTYRVVSVLTVLHQDWLNGKEYKCKVSNKALPAPIEKTISKAKGQPREPQVYTLPPSREEMTKNQVSLTCLVKGFYPSDIAVEWESNGQPENNYKTTPPVLDSDGSFFLYSKLTVDKSRWQQGNVFSCSVMHEALHNHYTQKSLSLSPGK

SEQ ID NO: 14 - DNA, 1368 bp, Artificial Sequence
  Description of Artificial Sequence: Synthetic polynucleotide
atggtcagctactgggacaccggggtcctgctgtgcgcgctgctcagctgtctgcttctcacaggatctagttcaggtatatttattagtgatacaggtagacctttcgtagagatgtacagtgaaatccccgaaattatacacatgactgaaggaagggagctcgtcattccctgccgggttacgtcacctaacatcactgttactttaaaaaagtttccacttgacactttgatccctgatggaaaacgcataatctgggacagtagaaagggcttcatcatatcaaatgcaacgtacaaagaaatagggcttctgacctgtgaagcaacagtcaatgggcatttgtataagacaaactatctcacacatcgacaaaccaatacaatcatagatgtcttcatcactgtgaaacatcgaaaacagcaggtgcttgaaaccgtagctggcaagcggtcttaccggctctctatgaaagtgaaggcatttccctcgccggaagttgtatggttaaaagatgggttacctgcgactgagaaatctgctcgctatttgactcgtggctactcgttaattatcaaggacgtaactgaagaggatgcagggaattatacaatcttgctgagcataaaacagtcaaatgtgtttaaaaacctcactgccactctaattgtcaatgtgaaacccgacaaaactcacacatgcccaccgtgcccagcacctgaactcctggggggaccgtcagtcttcctcttccccccaaaacccaaggacaccctcatgatctcccggacccctgaggtcacatgcgtggtggtggacgtgagccacgaagaccctgaggtcaagttcaactggtacgtggacggcgtggaggtgcataatgccaagacaaagccgcgggaggagcagtacaacagcacgtaccgtgtggtcagcgtcctcaccgtcctgcaccaggactggctgaatggcaaggagtacaagtgcaaggtctccaacaaagccctcccagcccccatcgagaaaaccatctccaaagccaaagggcagccccgagaaccacaggtgtacaccctgcccccatcccgggaggagatgaccaagaaccaggtcagcctgacctgcctggtcaaaggcttctatcccagcgacatcgccgtggagtgggagagcaatgggcagccggagaacaactacaagaccacgcctcccgtgctggactccgacggctccttcttcctctacagcaagctcaccgtggacaagagcaggtggcagcaggggaacgtcttctcatgctccgtgatgcacgaggctctgcacaaccactacacgcagaagagcctctccctgtctccgggtaaa